European Patent Application EP 4 324 840 A2, published February 21, 2024. Title: Alkaline stable Immunoglobulin-binding proteins. Applicant: Navigo Proteins GmbH. Application EP. The sequence listing filed with the application follows.

SEQUENCE LISTING (56 sequences)

SEQ ID NO: 1 - protein, 58 aa, synthetic construct
  REGION 1..58: note = generic sequence 1
  SITE 1: note = variant - may be replaced by V, N, Q, or P
  SITE 2: note = variant - may be replaced by D or Q
  SITE 3: note = variant - may be replaced by N or S
  SITE 4: note = variant - may be replaced byN
  SITE 5: note = variant - may be replaced by F
  SITE 6: note = variant - may be replaced by N, A, or S
  SITE 7: note = variant - may be replaced by E
  SITE 8: note = variant - may be replaced by E or A
  SITE 11: note = variant - may be replaced by N
  SITE 15: note = variant - may be replaced by Q
  SITE 16: note = variant - may be replaced by V
  SITE 18: note = variant - may be replaced by N
  SITE 19: note = variant - may be replaced by M
  SITE 21: note = variant - may be replaced by S or D
  SITE 23: note = variant - may be replaced by N
  SITE 24: note = variant - may be replaced by A
  SITE 25: note = variant - may be replaced by E
  SITE 28: note = variant - may be replaced by S or A
  SITE 29: note = variant - may be replaced by G
  SITE 40: note = variant - may be replaced by Q or T
  SITE 42: note = variant - may be replaced by A or T
  SITE 43: note = variant - may be replaced by N or S
  SITE 44: note = variant - may be replaced by V or L
  SITE 46: note = variant - may be replaced by A
  SITE 49: note = variant - may be replaced by Q
  SITE 52: note = variant - may be replaced by D or S
  SITE 53: note = variant - may be replaced by E
  SITE 54: note = variant - may be replaced by S
  SITE 58: note = variant - may be replaced by K
AAAKHDKDQQSAFYEILHLPNLTEDQRNAFIQSLKDDPSVSKEILGEAKKLNDAQAPP

SEQ ID NO: 2 - protein, 58 aa, synthetic construct; identical to SEQ ID NO: 1
  REGION 1..58: note = Generic sequence 2
  SITE 1: note = variant - may be replaced by N or P
  SITE 5: note = variant - may be replaced by F
  SITE 7: note = variant - may be replaced by E
  SITE 8: note = variant - may be replaced by E or A
  SITE 11: note = variant - may be replaced by N
  SITE 25: note = variant - may be replaced by E
  SITE 28: note = variant - may be replaced by S
  SITE 44: note = variant - may be replaced by V
  SITE 46: note = variant - may be replaced by A
  SITE 49: note = variant - may be replaced by Q
  SITE 54: note = variant - may be replaced by S
  SITE 58: note = variant - may be replaced by K

SEQ ID NO: 3 - protein, 58 aa, synthetic construct; identical to SEQ ID NO: 1
  REGION 1..58: note = parental protein IB14 1A/28N (IB14a)

SEQ ID NO: 4 - protein, 58 aa, synthetic construct
  REGION 1..58: note = parental protein IB27 1A
AAAKFDEAQQSAFYEILHLPNLTEEQRNAFIQSLKDDPSVSKEVLGEAQKLNDSQAPK

SEQ ID NO: 5 - protein, 58 aa, synthetic construct
  REGION 1..58: note = domain C
ADNKFNKEQQNAFYEILHLPNLTEEQRNGFIQSLKDDPSVSKEILAEAKKLNDAQAPK

SEQ ID NO: 6 - protein, 58 aa, synthetic construct [sequence omitted]

SEQ ID NO: 7 - protein, 58 aa, synthetic construct [sequence omitted]

SEQ ID NO: 8 - protein, 58 aa, synthetic construct [sequence omitted]

SEQ ID NO: 9 - protein, 58 aa, synthetic construct
  REGION 1..58: note = IB14 1I
IAAKHDKDQQSAFYEILHLPNLTEDQRSAFIQSLKDDPSVSKEILGEAKKLNDAQAPP

SEQ ID NO: 10 - protein, 58 aa, synthetic construct
  REGION 1..58: note = IB14 1A/28S (IB14b)
AAAKHDKDQQSAFYEILHLPNLTEDQRSAFIQSLKDDPSVSKEILGEAKKLNDAQAPP

SEQ ID NO: 11 - protein, 58 aa, synthetic construct
  REGION 1..58: note = IB14 11A
PAAKHDKDQQAAFYEILHLPNLTEDQRSAFIQSLKDDPSVSKEILGEAKKLNDAQAPP

SEQ ID NO: 12 - protein, 58 aa, synthetic construct
  REGION 1..58: note = IB14 11E
PAAKHDKDQQEAFYEILHLPNLTEDQRSAFIQSLKDDPSVSKEILGEAKKLNDAQAPP

SEQ ID NO: 13 - protein, 58 aa, synthetic construct
  REGION 1..58: note = IB14 11I
PAAKHDKDQQIAFYEILHLPNLTEDQRSAFIQSLKDDPSVSKEILGEAKKLNDAQAPP

SEQ ID NO: 14 - protein, 58 aa, synthetic construct
  REGION 1..58: note = IB14 1P 28S (IB14d)
PAAKHDKDQQSAFYEILHLPNLTEDQRSAFIQSLKDDPSVSKEILGEAKKLNDAQAPP

SEQ ID NO: 15 - protein, 58 aa, synthetic construct
  REGION 1..58: note = IB14 35R
PAAKHDKDQQSAFYEILHLPNLTEDQRSAFIQSLRDDPSVSKEILGEAKKLNDAQAPP

SEQ ID NO: 16 - protein, 58 aa, synthetic construct
  REGION 1..58: note = IB14 35I
PAAKHDKDQQSAFYEILHLPNLTEDQRSAFIQSLIDDPSVSKEILGEAKKLNDAQAPP

SEQ ID NO: 17 - protein, 58 aa, synthetic construct
  REGION 1..58: note = IB14 42L
PAAKHDKDQQSAFYEILHLPNLTEDQRSAFIQSLKDDPSVSLEILGEAKKLNDAQAPP

SEQ ID NO: 18 - protein, 58 aa, synthetic construct
  REGION 1..58: note = alkaline stable Ig binding domain cs14-1 (IB14 1I/11A/35R )
IAAKHDKDQQAAFYEILHLPNLTEDQRSAFIQSLRDDPSVSKEILGEAKKLNDAQAPP

SEQ ID NO: 19 - protein, 58 aa, synthetic construct
  REGION 1..58: note = alkaline stable Ig binding domain cs14-2 (IB14 1I/11A/35R/42L)
IAAKHDKDQQAAFYEILHLPNLTEDQRSAFIQSLRDDPSVSLEILGEAKKLNDAQAPP

SEQ ID NO: 20 - protein, 58 aa, synthetic construct
  REGION 1..58: note = alkaline stable Ig binding domain cs14-31I/11A/28N/35R/42L
IAAKHDKDQQAAFYEILHLPNLTEDQRNAFIQSLRDDPSVSLEILGEAKKLNDAQAPP

SEQ ID NO: 21 - protein, 58 aa, synthetic construct
  REGION 1..58: note = IB14 1P/28N (IB14c)
PAAKHDKDQQSAFYEILHLPNLTEDQRNAFIQSLKDDPSVSKEILGEAKKLNDAQAPP

SEQ ID NO: 22 - protein, 58 aa, synthetic construct
  REGION 1..58: note = IB27 1N
NAAKFDEAQQSAFYEILHLPNLTEEQRNAFIQSLKDDPSVSKEVLGEAQKLNDSQAPK

SEQ ID NO: 23 - protein, 53 aa, synthetic construct
  REGION 1..53: note = cs27 delNC
KFDEAQQAAFYEILHLPNLTEEQRNAFIQSLRDDPSVSLEVLGEAQKLNDSQA

SEQ ID NO: 24 - protein, 55 aa, synthetic construct
  REGION 1..55: note = cs27 delN
AFDEAQQAAFYEILHLPNLTEEQRNAFIQSLRDDPSVSLEVLGEAQKLNDSQAPK

SEQ ID NO: 25 - protein, 58 aa, synthetic construct
  REGION 1..58: note = parental protein IB25 1A
AAAKHDKDQQSAFYEILHLPNLTEDQRNAFIQSLKDDPSVSKEILAEAKKLNDAQAPK

SEQ ID NO: 26 - protein, 58 aa, synthetic construct
  REGION 1..58: note = alkaline stable Ig binding domain cs25 (IB25 1I/11A/35R/42L)
IAAKHDKDQQAAFYEILHLPNLTEDQRNAFIQSLRDDPSVSLEILAEAKKLNDAQAPK

SEQ ID NO: 27 - protein, 318 aa, synthetic construct
  REGION 1..318: note = cs17 delNC hexamer
KFDEAQQAAFYEILHLPNLTEEQRNAFIQSLRDDPSVSLEVLGEAQKLNDSQAKFDEAQQAAFYEILHLPNLTEEQRNAFIQSLRDDPSVSLEVLGEAQKLNDSQAKFDEAQQAAFYEILHLPNLTEEQRNAFIQSLRDDPSVSLEVLGEAQKLNDSQAKFDEAQQAAFYEILHLPNLTEEQRNAFIQSLRDDPSVSLEVLGEAQKLNDSQAKFDEAQQAAFYEILHLPNLTEEQRNAFIQSLRDDPSVSLEVLGEAQKLNDSQAKFDEAQQAAFYEILHLPNLTEEQRNAFIQSLRDDPSVSLEVLGEAQKLNDSQA

SEQ ID NO: 28 - protein, 290 aa, synthetic construct
  REGION 1..290: note = cs27 pentamer
IAAKFDEAQQAAFYEILHLPNLTEEQRNAFIQSLRDDPSVSLEVLGEAQKLNDSQAPKIAAKFDEAQQAAFYEILHLPNLTEEQRNAFIQSLRDDPSVSLEVLGEAQKLNDSQAPKIAAKFDEAQQAAFYEILHLPNLTEEQRNAFIQSLRDDPSVSLEVLGEAQKLNDSQAPKIAAKFDEAQQAAFYEILHLPNLTEEQRNAFIQSLRDDPSVSLEVLGEAQKLNDSQAPKIAAKFDEAQQAAFYEILHLPNLTEEQRNAFIQSLRDDPSVSLEVLGEAQKLNDSQAPK

SEQ ID NO: 29 - protein, 58 aa, synthetic construct
  REGION 1..58: note = alkaline stable Ig binding domain cs27-1 (IB27 1I/11A/35R)
IAAKFDEAQQAAFYEILHLPNLTEEQRNAFIQSLRDDPSVSKEVLGEAQKLNDSQAPK

SEQ ID NO: 30 - protein, 58 aa, synthetic construct
  REGION 1..58: note = alkaline stable Ig binding domain cs27-2 (IB27 I/11A/35R/42L)
IAAKFDEAQQAAFYEILHLPNLTEEQRNAFIQSLRDDPSVSLEVLGEAQKLNDSQAPK

SEQ ID NO: 31 - protein, 58 aa, synthetic construct
  REGION 1..58: note = alkaline stable Ig binding domain C 1I/11A/35R
IDNKFNKEQQAAFYEILHLPNLTEEQRNGFIQSLRDDPSVSKEILAEAKKLNDAQAPK

SEQ ID NO: 32 - protein, 58 aa, synthetic construct
  REGION 1..58: note = alkaline stable Ig binding domain C 1I/11A/35R/42L
IDNKFNKEQQAAFYEILHLPNLTEEQRNGFIQSLRDDPSVSLEILAEAKKLNDAQAPK

SEQ ID NO: 33 - protein, 58 aa, synthetic construct
  REGION 1..58: note = alkaline stable Ig binding domain B 1I/11A/35R
IDNKFNKEQQAAFYEILHLPNLNEEQRNGFIQSLRDDPSQSANLLAEAKKLNDAQAPK

SEQ ID NO: 34 - protein, 58 aa, synthetic construct
  REGION 1..58: note = alkaline stable Ig binding domain B 1I/11A/35R/42L
IDNKFNKEQQAAFYEILHLPNLNEEQRNGFIQSLRDDPSQSLNLLAEAKKLNDAQAPK

SEQ ID NO: 35 - protein, 58 aa, synthetic construct
  REGION 1..58: note = alkaline stable Ig binding domainZ 1I/11A/35R
IDNKFNKEQQAAFYEILHLPNLNEEQRNAFIQSLRDDPSQSANLLAEAKKLNDAQAPK

SEQ ID NO: 36 - protein, 58 aa, synthetic construct
  REGION 1..58: note = alkaline stable Ig binding domainZ 1I/11A/35R/42L
IDNKFNKEQQAAFYEILHLPNLNEEQRNAFIQSLRDDPSQSLNLLAEAKKLNDAQAPK

SEQ ID NO: 37 - protein, 58 aa, synthetic construct
  REGION 1..58: note = alkaline stable Ig binding domain domain Z/2 1I/11A/35R
IDAKFDKEQQAAFYEILHLPNLTEEQRNAFIQSLRDDPSQSLALLAEAKKLNDAQAPK

SEQ ID NO: 38 - protein, 58 aa, synthetic construct
  REGION 1..58: note = alkaline stable Ig binding domain Z/2 1I/11A/35R/42L
IDAKFDKEQQAAFYEILHLPNLTEEQRNAFIQSLRDDPSQSLNLLAEAKKLNDAQAPK

SEQ ID NO: 39 - protein, 79 aa, synthetic construct
  REGION 1..79: note = alkaline stable Ig binding domain cs14-3 with coupling sequenceand strep tag
IAAKHDKDQQAAFYEILHLPNLTEDQRNAFIQSLRDDPSVSLEILGEAKKLNDAQAPPASPAPSAPSACASWSHPQFEK

SEQ ID NO: 40 - protein, 79 aa, synthetic construct
  REGION 1..79: note = alkaline stable Ig binding domain cs27-2 with coupling sequenceand strep tag
IAAKFDEAQQAAFYEILHLPNLTEEQRNAFIQSLRDDPSVSLEVLGEAQKLNDSQAPKASPAPSAPSACASWSHPQFEK

SEQ ID NO: 41 - protein, 11 aa, synthetic construct
  REGION 1..11: note = coupling sequence
ASPAPSAPSAC

SEQ ID NO: 42 - protein, 58 aa, synthetic construct
  REGION 1..58: note = alkaline stable Ig binding domain cs74h1
IAAKFDEAQQAAFYEILHLPNLTEDQRNAFIQSLRDDPSVSLEILGEAKKLNDAQAPP

SEQ ID NO: 43 - protein, 58 aa, synthetic construct
  REGION 1..58: note = alkaline stable Ig binding domain cs74h2
IAAKFDEAQQAAFYEILHLPNLTEEQRNAFIQSLRDDPSVSLEILGEAKKLNDAQAPP

SEQ ID NO: 44 - protein, 58 aa, synthetic construct
  REGION 1..58: note = alkaline stable Ig binding domain cs47h3
IAAKHDKDQQAAFYEILHLPNLTEDQRNAFIQSLRDDPSVSLEVLGEAQKLNDSQAPK

SEQ ID NO: 45 - protein, 58 aa, synthetic construct
  REGION 1..58: note = alkaline stable Ig binding domain cs47h4
IAAKHDKDQQAAFYEILHLPNLTEEQRNAFIQSLRDDPSVSLEVLGEAQKLNDSQAPK

SEQ ID NO: 46 - protein, 8 aa, synthetic construct
  REGION 1..8: note = StrepTag
WSHPQFEK

SEQ ID NO: 47 - protein, 58 aa, synthetic construct
  REGION 1..58: note = parental protein IB74h1
AAAKFDEAQQSAFYEILHLPNLTEDQRNAFIQSLKDDPSVSKEILGEAKKLNDAQAPP

SEQ ID NO: 48 - protein, 58 aa, synthetic construct
  REGION 1..58: note = parental protein IB74h2
AAAKFDEAQQSAFYEILHLPNLTEEQRNAFIQSLKDDPSVSKEILGEAKKLNDAQAPP

SEQ ID NO: 49 - protein, 58 aa, synthetic construct
  REGION 1..58: note = parental protein IB47h3
AAAKHDKDQQSAFYEILHLPNLTEDQRNAFIQSLKDDPSVSKEVLGEAQKLNDSQAPK

SEQ ID NO: 50 - protein, 58 aa, synthetic construct
  REGION 1..58: note = parental protein IB47h4
AAAKHDKDQQSAFYEILHLPNLTEEQRNAFIQSLKDDPSVSKEVLGEAQKLNDSQAPK

SEQ ID NO: 51 - protein, 58 aa, synthetic construct; identical to SEQ ID NO: 1
  REGION 1..58: note = generic sequence including IB14 and IB27
  SITE 1: note = variant - may be replaced by N or P
  SITE 5: note = variant - may be replaced by F
  SITE 7: note = variant - may be replaced by E
  SITE 8: note = variant - may be replaced by A
  SITE 25: note = variant - may be replaced by E
  SITE 28: note = variant - may be replaced by S
  SITE 44: note = variant - may be replaced by V
  SITE 49: note = variant - may be replaced by Q
  SITE 54: note = variant - may be replaced by S
  SITE 58: note = variant - may be replaced by K

SEQ ID NO: 52 - protein, 58 aa, synthetic construct
  REGION 1..58: note = Generic sequence of preferred alkaline stable artifical IgGbinding proteins
  SITE 5: note = variant - may be replaced by F
  SITE 7: note = variant - may be replaced by E
  SITE 8: note = variant - may be replaced by A or E
  SITE 25: note = variant - may be replaced by E
  SITE 28: note = variant - may be replaced by S
  SITE 42: note = variant - may be replaced by L
  SITE 44: note = variant - may be replaced by V
  SITE 46: note = variant - may be replaced by A
  SITE 49: note = variant - may be replaced by Q
  SITE 54: note = variant - may be replaced by S
  SITE 58: note = variant - may be replaced by K
IAAKHDKDQQAAFYEILHLPNLTEDQRNAFIQSLRDDPSVSKEILGEAKKLNDAQAPP

SEQ ID NO: 53 - protein, 58 aa, synthetic construct
  REGION 1..58: note = cs27 46C
IAAKFDEAQQAAFYEILHLPNLTEEQRNAFIQSLRDDPSVSLEVLCEAQKLNDSQAPK

SEQ ID NO: 54 - protein, 58 aa, synthetic construct
  REGION 1..58: note = cs14 43C
IAAKHDKDQQAAFYEILHLPNLTEDQRNAFIQSLRDDPSVSLCILGEAKKLNDAQAPP

SEQ ID NO: 55 - protein, 174 aa, synthetic construct
  REGION 1..174: note = cs27 tetramer
IAAKFDEAQQAAFYEILHLPNLTEEQRNAFIQSLRDDPSVSLEVLGEAQKLNDSQAPKIAAKFDEAQQAAFYEILHLPNLTEEQRNAFIQSLRDDPSVSLEVLGEAQKLNDSQAPKIAAKFDEAQQAAFYEILHLPNLTEEQRNAFIQSLRDDPSVSLEVLGEAQKLNDSQAPK

SEQ ID NO: 56 - protein, 5 aa, synthetic construct
  REGION 1..5: note = coupling sequence
GGGSC